European Patent Specification EP 3 894 593 B1, published October 2, 2024. Title: DIRECT OLIGONUCLEOTIDE SYNTHESIS ON CELLS AND BIOMOLECULES. Applicant: DNA SCRIPT. The sequence listing filed with the application follows.

SEQUENCE LISTING (18 sequences)

SEQ ID NO: 1 - protein, 510 aa, ARTIFICIAL SEQUENCE
  TDT enzyme
MDPLQAVHLGPRKKRPRQLGTPVASTPYDIRFRDLVLFILEKKMGTTRRAFLMELARRKGFRVENELSDSVTHIVAENNSGSDVLEWLQLQNIKASSELELLDISWLIECMGAGKPVEMMGRHQLVVNRNSSPSPVPGSQNVPAPAVKKISQYACQRRTTLNNYNQLFTDALDILAENDELRENEGSCLAFMRASSVLKSLPFPITSMKDTEGIPCLGDKVKSIIEGIIEDGESSEAKAVLNDERYKSFKLFTSVFGVGLKTAEKWFRMGFRTLSKIQSDKSLRFTQMQKAGFLYYEDLVSCVNRPEAEAVSMLVKEAVVTFLPDALVTMTGGFRRGKMTGHDVDFLITSPEATEDEEQQLLHKVTDFWKQQGLLLYCDILESTFEKFKQPSRKVDALDHFQKCFLILKLDHGRVHSEKSGQQEGKGWKAIRVDLVMCPYDRRAFALLGWTGSRQFERDLRRYATHERKMMLDNHALYDRTKRVFLEAESEEEIFAHLGLDYIEPWERNA

SEQ ID NO: 2 - protein, 381 aa, ARTIFICIAL SEQUENCE
  truncated mouse sequence
NSSPSPVPGSQNVPAPAVKKISQYACQRRTTLNNYNQLFTDALDILAENDELRENEGSCLAFMRASSVLKSLPFPITSMKDTEGIPCLGDKVKSIIEGIIEDGESSEAKAVLNDERYKSFKLFTSVFGVGLKTAEKWFRMGFRTLSKIQSDKSLRFTQMQKAGFLYYEDLVSCVNRPEAEAVSMLVKEAVVTFLPDALVTMTGGFRRGKMTGHDVDFLITSPEATEDEEQQLLHKVTDFWKQQGLLLYCDILESTFEKFKQPSRKVDALDHFQKCFLILKLDHGRVHSEKSGQQEGKGWKAIRVDLVMCPYDRRAFALLGWTGSRQFERDLRRYATHERKMMLDNHALYDRTKRVFLEAESEEEIFAHLGLDYIEPWERNA

SEQ ID NO: 3 - protein, 380 aa, ARTIFICIAL SEQUENCE
  Bovine truncated (catalytic domain):
DYSATPNPGFQKTPPLAVKKISQYACQRKTTLNNYNHIFTDAFEILAENSEFKENEVSYVTFMRAASVLKSLPFTIISMKDTEGIPCLGDKVKCIIEEIIEDGESSEVKAVLNDERYQSFKLFTSVFGVGLKTSEKWFRMGFRSLSKIMSDKTLKFTKMQKAGFLYYEDLVSCVTRAEAEAVGVLVKEAVWAFLPDAFVTMTGGFRRGKKIGHDVDFLITSPGSAEDEEQLLPKVINLWEKKGLLLYYDLVESTFEKFKLPSRQVDTLDHFQKCFLILKLHHQRVDSSKSNQQEGKTWKAIRVDLVMCPYENRAFALLGWTGSRQFERDIRRYATHERKMMLDNHALYDKTKRVFLKAESEEEIFAHLGLDYIEPWERNA

SEQ ID NO: 4 - protein, 380 aa, ARTIFICIAL SEQUENCE
  Human truncated
DYSDSTNPGPPKTPPIAVQKISQYACQRRTTLNNCNQIFTDAFDILAENCEFRENEDSCVTFMRAASVLKSLPFTIISMKDTEGIPCLGSKVKGIIEEIIEDGESSEVKAVLNDERYQSFKLFTSVFGVGLKTSEKWFRMGFRTLSKVRSDKSLKFTRMQKAGFLYYEDLVSCVTRAEAEAVSVLVKEAVWAFLPDAFVTMTGGFRRGKKMGHDVDFLITSPGSTEDEEQLLQKVMNLWEKKGLLLYYDLVESTFEKLRLPSRKVDALDHFQKCFLIFKLPRQRVDSDQSSWQEGKTWKAIRVDLVLCPYERRAFALLGWTGSRQFERDLRRYATHERKMILDNHALYDKTKRIFLKAESEEEIFAHLGLDYIEPWERNA

SEQ ID NO: 5 - protein, 376 aa, ARTIFICIAL SEQUENCE
  Chicken 1 truncated
QYPTLKTPESEVSSFTASKVSQYSCQRKTTLNNCNKKFTDAFEIMAENYEFKENEIFCLEFLRAASVLKSLPFPVTRMKDIQGLPCMGDRVRDVIEEIIEEGESSRAKDVLNDERYKSFKEFTSVFGVGVKTSEKWFRMGLRTVEEVKADKTLKLSKMQRAGFLYYEDLVSCVSKAEADAVSSIVKNTVCTFLPDALVTITGGFRRGKKIGHDIDFLITSPGQREDDELLHKGLLLYCDIIESTFVKEQIPSRHVDAMDHFQKCFAILKLYQPRVDNSSYNMSKKCDMAEVKDWKAIRVDLVITPFEQYAYALLGWTGSRQFGRDLRRYATHERKMMLDNHALYDKRKRVFLKAGSEEEIFAHLGLDYVEPWERNA

SEQ ID NO: 6 - protein, 387 aa, ARTIFICIAL SEQUENCE
  Possum truncated
SANPDPTAGTLNILPPTTKTISQYACQRRTTINNHNQRFTDAFEILAKNYEFKENDDTCLTFMRAISVLKCLPFEVVSLKDTEGLPWIGDEVKGIMEEIIEDGESLEVQAVLNDERYQSFKLFTSVFGVGLKTADKWYRMGFRTLNKIRSDKTLKLTKMQKAGLCYYEDLIDCVSKAEADAVSLLVQDAVWTFLPDALVTITGGFRRGKEFGHDVDFLITSPGAEKEQEDQLLQKVTNLWKKQGLLLYCDLIESTFEDLKLPSRKIDALDHFQKCFLILKLYHHKEDKRKWEMPTGSNESEAKSWKAIRVDLVVCPYDRYAFALLGWSGSRQFERDLRRYATHEKKMMLDNHALYDKTKKIFLKAKSEEEIFAHLGLEYIQPSERNA

SEQ ID NO: 7 - protein, 381 aa, ARTIFICIAL SEQUENCE
  New truncated shrew
DCPASHDSSPQKTESAAVQKISQYACQRRTTLNNHNHIFTDAFEILAENCEFRENEGSYVTYMRAASVLKSLPFSIISMKDTEGIPCLADKVKCVIEEIIEDGESSEVKAVLNDERYKSFKLFTSVFGVGLKTAEKWFRLGFRTLSGIMNDKTLKLTHMQKAGFLYYEDLVSCVTRAEAEAVGVLVKEAVWAFLPDAIVTMTGGFRRGKKVGHDVDFLITSPEATEEQEQQLLHKVITFWEKEGLLLYCDLYESTFEKLKMPSRKVDALDHFQKCFLILKLHRECVDDGTSSQLQGKTWKAIRVDLVVCPYECRAFALLGWTGSPQFERDLRRYATHERKMMLDNHALYDKTKRKFLSADSEEDIFAHLGLDYIEPWERNA

SEQ ID NO: 8 - protein, 387 aa, ARTIFICIAL SEQUENCE
  Python truncated
EKYQLPEDEDRSVTSDLDRDSISEYACQRRTTLKNYNQKFTDAFEILAENYEFNENKGFCTAFRRAASVLKCLPFTIVQVHDIEGVPWMGKQVKGIIEDIIEEGESSKVKAVLDNENYRSVKLFTSVFGVGLKTSDKWYRMGLRTLEEVKRDKNLKLTRMQKAGFLHYDDLTSCVSKAEADAASLIVQDVVWKIVPNAIVTIAGGFRRGKQTGHDVDFLITVPGSKQEEEELLHTVIDIWKKQELLLYYDLIESTFEDTKLPSRKVDALDHFQKCFAILKVHKEREDKGNSIRSKAFSEEEIKDWKAIRVDLVVVPFEQYAFALLGWTGSTQFERDLRRYATHEKKMMLDNHALYDKTKKIFLNAASEEEIFAHLGLDYLEPWERNA

SEQ ID NO: 9 - protein, 381 aa, ARTIFICIAL SEQUENCE
  truncated dog
DYTASPNPELQKTLPVAVKKISQYACQRRTTLNNYNNVFTDAFEVLAENYEFRENEVFSLTFMRAASVLKSLPFTIISMKDTEGIPCLGDQVKCIIEEIIEDGESSEVKAVLNDERYQSFKLFTSVFGVGLKTSEKWFRMGFRTLSKIKSDKSLKFTPMQKAGFLYYEDLVSCVTRAEAEAVGVLVKEAVGAFLPDAFVTMTGGFRRGKKMGHDVDFLITSPGSTDEDEEQLLPKVINLWERKGLLLYCDLVESTFEKLKLPSRKVDALDHFQKCFLILKLHHQRVDGGKCSQQEGKTWKAIRVDLVMCPYERRAFALLGWTGSRQFERDLRRYASHERKMILDNHALYDKTKKIFLKAESEEEIFAHLGLDYIEPWERNA

SEQ ID NO: 10 - protein, 382 aa, ARTIFICIAL SEQUENCE
  TRUNC MOLE
GDCPASHDSSPQKTESAAVQKISQYACQRRTTLNNHNHIFTDAFEILAENCEFRENEGSYVTYMRAASVLKSLPFSIISMKDTEGIPCLADKVKCVIEEIIEDGESSEVKAVLNDERYKSFKLFTSVFGVGLKTAEKWFRLGFRTLSGIMNDKTLKLTHMQKAGFLYYEDLVSCVTRAEAEAVGVLVKEAVWAFLPDAIVTMTGGFRRGKKVGHDVDFLITSPEATEEQEQQLLHKVITFWEKEGLLLYCDLYESTFEKLKMPSRKVDALDHFQKCFLILKLHRECVDDGTSSQLQGKTWKAIRVDLVVCPYECRAFALLGWTGSPQFERDLRRYATHERKMMLDNHALYDKTKRKFLSADSEEDIFAHLGLDYIEPWERNA

SEQ ID NO: 11 - protein, 379 aa, ARTIFICIAL SEQUENCE
  Pika trunk
EYSANPSPGPQATPAVYKISQYACQRRTTLNNHNHIFTDAFEILAENYEFKENEGCYVTYMRAASVLKSLPFTIVSMKDTEGIPCLEDKVKSIMEEIIEEGESSEVKAVLSDERYQCFKLFTSVFGVGLKTSEKWFRMGFRSLSNIRLDKSLKFTQMQKAGFRYYEDIVSCVTRAEAEAVDVLVNEAVRAFLPDAFITMTGGFRRGKKIGHDVDFLITSPELTEEDEQQLLHKVMNLWEKKGLLLYHDLVESTFEKLKQPSRKVDALDHFQKCFLIFKLYHERVGGDRCRQPEGKDWKAIRVDLVMCPYECHAFALLGWTGSRQFERDLRRYASHERKMILDNHALYDKTKRVFLQAENEEEIFAHLGLDYIEPWERNA

SEQ ID NO: 12 - protein, 384 aa, ARTIFICIAL SEQUENCE
  TRUNC HEDGEHOG
DASFGSNPGSQNTPPLAIKKISQYACQRRTSLNNCNHIFTDALDILAENHEFRENEVSCVAFMRAASVLKSLPFTIISMKDTKGIPCLGDKAKCVIEEIIEDGESSEVKAILNDERYQSFKLFTSVFGVGLKTSEKWFRMGFRTLNKIMSDKTLKLTRMQKAGFLYYEDLVSCVAKAEADAVSVLVQEAVWAFLPDAMVTMTGGFRRGKKLGHDVDFLITSPGATEEEEQQLLPKVINFWERKGLLLYHDLVESTFEKLKLPSRKVDALDHFQKCFLILKLHLQHVNGVGNSKTGQQEGKNWKAIRVDLVMCPYERRAFALLGWTGSRQFERDLRRFATHERKMMLDNHALYDKTKRIFLKAESEEEIFAHLGLDYIDPWERNA

SEQ ID NO: 13 - protein, 381 aa, ARTIFICIAL SEQUENCE
  truncated tree shrew
DHSTSPSPGPQKTPALAVQKISQYACQRRTTLNNCNRVFTDAFETLAENYEFRENEDSSVIFLRAASVLRSLPFTITSMRDTEGLPCLGDKVKCVIEEIIEDGESSEVNAVLNDERYKSFKLFTSVFGVGLKTSEKWFRMGFRTLSRVRSDKSLHLTRMQQAGFLYYEDLASCVTRAEAEAVGVLVKEAVGAFLPDALVTITGGFRRGKKTGHDVDFLITSPGSTEEKEEELLQKVLNLWEKKGLLLYYDLVESTFEKLKTPSRKVDALDHFPKCFLILKLHHQRVDGDKPSQQEGKSWKAIRVDLVMCPYERHAFALLGWTGSRQFERDLRRYATHERKMMLDNHALYDKTKRVFLKAESEEDIFAHLGLDYIEPWERNA

SEQ ID NO: 14 - protein, 394 aa, ARTIFICIAL SEQUENCE
  TRUNCATED PLATYPUS
LTNSAPINCMTETPSLATKQVSQYACERRTTLNNCNQKFTDAFEILAKDFEFRENEGICLAFMRAISVLKCLPFTIVRMKDIEGVPWLGDQVKSIIEEIIEDGESSSVKAVLNDERYRSFQLFNSVFEVGLTDNGENGIARGFQTLNEVITDENISLTKTTLSTSLWNYLPGFLYYEDLVSCVAKEEADAVYLIVKEAVRAFLPEALVTLTGGFRRGKKIGHDVDFLISDPESGQDEQLLPNIIKLWEKQELLLYYDLVESTFEKTKIPSRKVDAMDHFQKCFLILKLHHQKVDSGRYKPPPESKNHEAKNWKAIRVDLVMCPFEQYAYALLGWTGSRQFERDLRRYATHEKKMMLDNHALYDKTKKIFLKAESEEDIFTHLGLDYIEPWERNA

SEQ ID NO: 15 - protein, 384 aa, ARTIFICIAL SEQUENCE
  TRUNCATED JERBOA
SSELELLDVSWLIECMGAGKPVEMTGRHQLVKQTFCLPGFILQDAFDILAENCEFRENEASCVEFMRAASVLKSLPFPIISVKDTEGIPWLGGKVKCVIEEIIEDGESSEVKALLNDERYKSFKLFTSVFGVGLKTAERWFRMGFRTLSTVKLDKSLTFTRMQKAGFLHYEDLVSCVTRAEAEAVSVLVQQAVVAFLPDALVSMTGGFRRGKKIGHDVDFLITSPEATEEEEQQLLHKVTNFWEQKGLLLYCDHVESTFEKCKLPSRKVDALDHFQKCFLILKLYRERVDSVKSSQQEGKGWKAIRVDLVMCPYECRAFALLGWTGSRQFERDLRRYATHERKMRLDNHALYDKTKRVFLKAESEEEIFAHLGLEYIEPLERNA

SEQ ID NO: 16 - DNA, 32 bp, ARTIFICIAL SEQUENCE
  Exemplary cDNA produced in a method of the invention (Fig. 1B)
  misc_feature (8)..(32): n is a, c, g, t or u
tttttttnnnnnnnnnnnnnnnnnnnnnnnnn

SEQ ID NO: 17 - DNA, 15 bp, ARTIFICIAL SEQUENCE
  Exemplary cDNA produced in process of Fig. 4A
  misc_feature (15)..(15): n is a, c, g, t or u
ttttttttttttttn

SEQ ID NO: 18 - DNA, 13 bp, ARTIFICIAL SEQUENCE
  Antibody barcode
  misc_feature (8)..(13): n is a, c, g, t or u
aaaaaaannnnnn